European Patent Application EP 4 218 751 A2, published August 2, 2023. Title: DIETARY PRODUCT DEVOID OF AT LEAST TWO NON ESSENTIAL AMINO ACIDS. Applicant: Cancer Research Technology Ltd. Application EP. The sequence listing filed with the application follows.

SEQUENCE LISTING (12 sequences)

SEQ ID NO: 1 - DNA, 21 bp, synthetic construct
  misc_feature 1..21: note = Forward Primer Mouse PSAT1
  source 1..21: mol_type = other DNA
tggcctcggcagaattggaag

SEQ ID NO: 2 - DNA, 22 bp, synthetic construct
  misc_feature 1..22: note = Reverse Primer Mouse PHGDH
  source 1..22: mol_type = other DNA
tgtcattcagcaagcctgtggt

SEQ ID NO: 3 - DNA, 24 bp, synthetic construct
  misc_feature 1..24: note = Forward Primer Mouse PSAT1
  source 1..24: mol_type = other DNA
gatgaacatcccatttcgcattgg

SEQ ID NO: 4 - DNA, 24 bp, synthetic construct
  misc_feature 1..24: note = Reverse Primer Mouse PSAT1
  source 1..24: mol_type = other DNA
gcgttatacagagaggcacgaatg

SEQ ID NO: 5 - DNA, 24 bp, synthetic construct
  misc_feature 1..24: note = Forward Primer Mouse PSPH
  source 1..24: mol_type = other DNA
gagatggagctacggacatggaag

SEQ ID NO: 6 - DNA, 24 bp, synthetic construct
  misc_feature 1..24: note = Reverse Primer Mouse PSPH
  source 1..24: mol_type = other DNA
ctcctccagttctcccagcagctc

SEQ ID NO: 7 - DNA, 25 bp, synthetic construct
  misc_feature 1..25: note = MTAP_gRNA_1F sequence ONE
  source 1..25: mol_type = other DNA
caccggttttgccccaaaacgagag

SEQ ID NO: 8 - DNA, 25 bp, synthetic construct
  misc_feature 1..25: note = MTAP_gRNA_1R sequence ONE
  source 1..25: mol_type = other DNA
aaacctctcgttttggggcaaaacc

SEQ ID NO: 9 - DNA, 25 bp, synthetic construct
  misc_feature 1..25: note = MTAP_gRNA_2F sequence TWO
  source 1..25: mol_type = other DNA
caccggcctggtagttgacctttga

SEQ ID NO: 10 - DNA, 25 bp, synthetic construct
  misc_feature 1..25: note = MTAP_gRNA_2R sequence TWO
  source 1..25: mol_type = other DNA
aaactcaaaggtcaactaccaggcc

SEQ ID NO: 11 - DNA, 25 bp, synthetic construct
  misc_feature 1..25: note = NTC_gRNA_1F
  source 1..25: mol_type = other DNA
caccgaaaatagcagtaaactcaac

SEQ ID NO: 12 - DNA, 25 bp, synthetic construct
  misc_feature 1..25: note = NTC_gRNA_1R
  source 1..25: mol_type = other DNA
aaacgttgagtttactgctattttc